European Patent Application EP 4 763 988 A1, published June 24, 2026. Title: 特异性结合CDCP1的单域抗体及其应用. Applicant: 明慧医药（杭州）有限公司. The sequence listing filed with the application follows.

SEQUENCE LISTING (51 sequences)

SEQ ID NO: 1 - protein, 5 aa, synthetic construct
ANGMV

SEQ ID NO: 2 - protein, 16 aa, synthetic construct
VISSSGSTNYADSVKG

SEQ ID NO: 3 - protein, 7 aa, synthetic construct
AHYGQTY

SEQ ID NO: 4 - protein, 7 aa, synthetic construct
GSDVSAN

SEQ ID NO: 5 - protein, 5 aa, synthetic construct
SSSGS

SEQ ID NO: 6 - protein, 7 aa, synthetic construct
AHYGQTY

SEQ ID NO: 7 - protein, 8 aa, synthetic construct
GSDVSANG

SEQ ID NO: 8 - protein, 7 aa, synthetic construct
ISSSGST

SEQ ID NO: 9 - protein, 9 aa, synthetic construct
GVAHYGQTY

SEQ ID NO: 10 - protein, 115 aa, synthetic construct
QLQLVESGGGLVQPGGSLRLSCAASGSDVSANGMVWHRQAPGKQREWVAVISSSGSTNYADSVKGRFTISRDSDKNTMYLQMNNLKPEDTAVYLCGVAHYGQTYWGKGTLVTVSS

SEQ ID NO: 11 - protein, 115 aa, synthetic construct
EVQLVESGGGLVQPGGSLRLSCAASGSDVSANGMVWHRQAPGKQREWVAVISSSGSTNYADSVKGRFTISRDSDKNTMYLQMNSLRPEDTAVYLCGVAHYGQTYWGKGTLVTVSS

SEQ ID NO: 12 - protein, 115 aa, synthetic construct
EVQLVESGGGLVQPGGSLRLSCAASGSDVSANGMVWHRQAPGKGREWVAVISSSGSTNYADSVKGRFTISRDSDKNTMYLQMNSLRPEDTAVYLCGVAHYGQTYWGKGTLVTVSS

SEQ ID NO: 13 - protein, 115 aa, synthetic construct
EVQLVESGGGLVQPGGSLRLSCAASGSDVSANGMVWHRQAPGKGREWVAVISSSGSTNYADSVKGRFTISRDNSKNTMYLQMNSLRPEDTAVYLCGVAHYGQTYWGKGTLVTVSS

SEQ ID NO: 14 - protein, 115 aa, synthetic construct
EVQLVESGGGLVQPGGSLRLSCAASGSDVSANGMVWHRQAPGKGREWVAVISSSGSTNYADSVKGRFTISRDNSKNTMYLQMNSLRPEDTAVYYCGVAHYGQTYWGKGTLVTVSS

SEQ ID NO: 15 - protein, 115 aa, synthetic construct
EVQLVESGGGLVQPGGSLRLSCAASGSDVSANGMVWHRQAPGKGREWVAVISSSGSTNYADSVKGRFTISRDSDKNTMYLQMNSLRPEDTAVYYCGVAHYGQTYWGKGTLVTVSS

SEQ ID NO: 16 - protein, 115 aa, synthetic construct
EVQLVESGGGLVQPGGSLRLSCAASGSDVSANGMVWHRQAPGKQREWVAVISSSGSTNYADSVKGRFTISRDNSKNTMYLQMNSLRPEDTAVYLCGVAHYGQTYWGKGTLVTVSS

SEQ ID NO: 17 - protein, 115 aa, synthetic construct
EVQLVESGGGLVQPGGSLRLSCAASGSDVSANGMVWHRQAPGKQREWVAVISSSGSTNYADSVKGRFTISRDNSKNTMYLQMNSLRPEDTAVYYCGVAHYGQTYWGKGTLVTVSS

SEQ ID NO: 18 - protein, 115 aa, synthetic construct
EVQLVESGGGLVQPGGSLRLSCAASGSDVSANGMVWHRQAPGKQREWVAVISSSGSTNYADSVKGRFTISRDSDKNTMYLQMNSLRPEDTAVYYCGVAHYGQTYWGKGTLVTVSS

SEQ ID NO: 19 - protein, 115 aa, synthetic construct
QLQLVESGGGLVQPGGSLRLSCAASGSDVSANGMVWHRQAPGKQREWVAVISSSGSTNYADSVKGRFTISRDSDKNTMYLQMNSLRPEDTAVYLCGVAHYGQTYWGKGTLVTVSS

SEQ ID NO: 20 - protein, 115 aa, synthetic construct
EVQLVESGGGLVQPGGSLRLSCAASGSDVSANGMVWHRQAPGKQREWVAVISSSGSTNYADSVKGRFTISRDSDKNTMYLQMNNLKPEDTAVYLCGVAHYGQTYWGKGTLVTVSS

SEQ ID NO: 21 - protein, 115 aa, synthetic construct
QLQLVESGGGLVQPGGSLRLSCAASGSDVSANGMVWHRQAPGKGREWVAVISSSGSTNYADSVKGRFTISRDSDKNTMYLQMNSLRPEDTAVYLCGVAHYGQTYWGKGTLVTVSS

SEQ ID NO: 22 - protein, 115 aa, synthetic construct
QLQLVESGGGLVQPGGSLRLSCAASGSDVSANGMVWHRQAPGKGREWVAVISSSGSTNYADSVKGRFTISRDNSKNTMYLQMNSLRPEDTAVYLCGVAHYGQTYWGKGTLVTVSS

SEQ ID NO: 23 - protein, 115 aa, synthetic construct
QLQLVESGGGLVQPGGSLRLSCAASGSDVSANGMVWHRQAPGKGREWVAVISSSGSTNYADSVKGRFTISRDNSKNTMYLQMNSLRPEDTAVYYCGVAHYGQTYWGKGTLVTVSS

SEQ ID NO: 24 - protein, 115 aa, synthetic construct
QLQLVESGGGLVQPGGSLRLSCAASGSDVSANGMVWHRQAPGKGREWVAVISSSGSTNYADSVKGRFTISRDSDKNTMYLQMNSLRPEDTAVYYCGVAHYGQTYWGKGTLVTVSS

SEQ ID NO: 25 - protein, 115 aa, synthetic construct
QLQLVESGGGLVQPGGSLRLSCAASGSDVSANGMVWHRQAPGKQREWVAVISSSGSTNYADSVKGRFTISRDNSKNTMYLQMNSLRPEDTAVYLCGVAHYGQTYWGKGTLVTVSS

SEQ ID NO: 26 - protein, 115 aa, synthetic construct
QLQLVESGGGLVQPGGSLRLSCAASGSDVSANGMVWHRQAPGKQREWVAVISSSGSTNYADSVKGRFTISRDNSKNTMYLQMNSLRPEDTAVYYCGVAHYGQTYWGKGTLVTVSS

SEQ ID NO: 27 - protein, 115 aa, synthetic construct
QLQLVESGGGLVQPGGSLRLSCAASGSDVSANGMVWHRQAPGKQREWVAVISSSGSTNYADSVKGRFTISRDSDKNTMYLQMNSLRPEDTAVYYCGVAHYGQTYWGKGTLVTVSS

SEQ ID NO: 28 - protein, 232 aa, synthetic construct
EPKSCDKTHTCPPCPAPEAAGGPSVFLFPPKPKDTLMISRTPEVTCVVVDVSHEDPEVKFNWYVDGVEVHNAKTKPREEQYNSTYRVVSVLTVLHQDWLNGKEYKCKVSNKALPAPIEKTISKAKGQPREPQVYTLPPSREEMTKNQVSLTCLVKGFYPSDIAVEWESNGQPENNYKTTPPVLDSDGSFFLYSKLTVDKSRWQQGNVFSCSVMHEALHNHYTQKSLSLSPGK

SEQ ID NO: 29 - protein, 232 aa, synthetic construct
EPKSSDKTHTCPPCPAPEAAGGPSVFLFPPKPKDTLMISRTPEVTCVVVDVSHEDPEVKFNWYVDGVEVHNAKTKPREEQYNSTYRVVSVLTVLHQDWLNGKEYKCKVSNKALPAPIEKTISKAKGQPREPQVYTLPPSREEMTKNQVSLTCLVKGFYPSDIAVEWESNGQPENNYKTTPPVLDSDGSFFLYSKLTVDKSRWQQGNVFSCSVMHEALHNHYTQKSLSLSPGK

SEQ ID NO: 30 - protein, 347 aa, synthetic construct
QLQLVESGGGLVQPGGSLRLSCAASGSDVSANGMVWHRQAPGKQREWVAVISSSGSTNYADSVKGRFTISRDSDKNTMYLQMNNLKPEDTAVYLCGVAHYGQTYWGKGTLVTVSSEPKSCDKTHTCPPCPAPEAAGGPSVFLFPPKPKDTLMISRTPEVTCVVVDVSHEDPEVKFNWYVDGVEVHNAKTKPREEQYNSTYRVVSVLTVLHQDWLNGKEYKCKVSNKALPAPIEKTISKAKGQPREPQVYTLPPSREEMTKNQVSLTCLVKGFYPSDIAVEWESNGQPENNYKTTPPVLDSDGSFFLYSKLTVDKSRWQQGNVFSCSVMHEALHNHYTQKSLSLSPGK

SEQ ID NO: 31 - protein, 347 aa, synthetic construct
EVQLVESGGGLVQPGGSLRLSCAASGSDVSANGMVWHRQAPGKQREWVAVISSSGSTNYADSVKGRFTISRDSDKNTMYLQMNSLRPEDTAVYLCGVAHYGQTYWGKGTLVTVSSEPKSSDKTHTCPPCPAPEAAGGPSVFLFPPKPKDTLMISRTPEVTCVVVDVSHEDPEVKFNWYVDGVEVHNAKTKPREEQYNSTYRVVSVLTVLHQDWLNGKEYKCKVSNKALPAPIEKTISKAKGQPREPQVYTLPPSREEMTKNQVSLTCLVKGFYPSDIAVEWESNGQPENNYKTTPPVLDSDGSFFLYSKLTVDKSRWQQGNVFSCSVMHEALHNHYTQKSLSLSPGK

SEQ ID NO: 32 - protein, 347 aa, synthetic construct
EVQLVESGGGLVQPGGSLRLSCAASGSDVSANGMVWHRQAPGKGREWVAVISSSGSTNYADSVKGRFTISRDSDKNTMYLQMNSLRPEDTAVYLCGVAHYGQTYWGKGTLVTVSSEPKSSDKTHTCPPCPAPEAAGGPSVFLFPPKPKDTLMISRTPEVTCVVVDVSHEDPEVKFNWYVDGVEVHNAKTKPREEQYNSTYRVVSVLTVLHQDWLNGKEYKCKVSNKALPAPIEKTISKAKGQPREPQVYTLPPSREEMTKNQVSLTCLVKGFYPSDIAVEWESNGQPENNYKTTPPVLDSDGSFFLYSKLTVDKSRWQQGNVFSCSVMHEALHNHYTQKSLSLSPGK

SEQ ID NO: 33 - protein, 347 aa, synthetic construct
EVQLVESGGGLVQPGGSLRLSCAASGSDVSANGMVWHRQAPGKGREWVAVISSSGSTNYADSVKGRFTISRDNSKNTMYLQMNSLRPEDTAVYLCGVAHYGQTYWGKGTLVTVSSEPKSSDKTHTCPPCPAPEAAGGPSVFLFPPKPKDTLMISRTPEVTCVVVDVSHEDPEVKFNWYVDGVEVHNAKTKPREEQYNSTYRVVSVLTVLHQDWLNGKEYKCKVSNKALPAPIEKTISKAKGQPREPQVYTLPPSREEMTKNQVSLTCLVKGFYPSDIAVEWESNGQPENNYKTTPPVLDSDGSFFLYSKLTVDKSRWQQGNVFSCSVMHEALHNHYTQKSLSLSPGK

SEQ ID NO: 34 - protein, 347 aa, synthetic construct
EVQLVESGGGLVQPGGSLRLSCAASGSDVSANGMVWHRQAPGKGREWVAVISSSGSTNYADSVKGRFTISRDNSKNTMYLQMNSLRPEDTAVYYCGVAHYGQTYWGKGTLVTVSSEPKSSDKTHTCPPCPAPEAAGGPSVFLFPPKPKDTLMISRTPEVTCVVVDVSHEDPEVKFNWYVDGVEVHNAKTKPREEQYNSTYRVVSVLTVLHQDWLNGKEYKCKVSNKALPAPIEKTISKAKGQPREPQVYTLPPSREEMTKNQVSLTCLVKGFYPSDIAVEWESNGQPENNYKTTPPVLDSDGSFFLYSKLTVDKSRWQQGNVFSCSVMHEALHNHYTQKSLSLSPGK

SEQ ID NO: 35 - protein, 347 aa, synthetic construct
EVQLVESGGGLVQPGGSLRLSCAASGSDVSANGMVWHRQAPGKGREWVAVISSSGSTNYADSVKGRFTISRDSDKNTMYLQMNSLRPEDTAVYYCGVAHYGQTYWGKGTLVTVSSEPKSSDKTHTCPPCPAPEAAGGPSVFLFPPKPKDTLMISRTPEVTCVVVDVSHEDPEVKFNWYVDGVEVHNAKTKPREEQYNSTYRVVSVLTVLHQDWLNGKEYKCKVSNKALPAPIEKTISKAKGQPREPQVYTLPPSREEMTKNQVSLTCLVKGFYPSDIAVEWESNGQPENNYKTTPPVLDSDGSFFLYSKLTVDKSRWQQGNVFSCSVMHEALHNHYTQKSLSLSPGK

SEQ ID NO: 36 - protein, 347 aa, synthetic construct
EVQLVESGGGLVQPGGSLRLSCAASGSDVSANGMVWHRQAPGKQREWVAVISSSGSTNYADSVKGRFTISRDNSKNTMYLQMNSLRPEDTAVYLCGVAHYGQTYWGKGTLVTVSSEPKSSDKTHTCPPCPAPEAAGGPSVFLFPPKPKDTLMISRTPEVTCVVVDVSHEDPEVKFNWYVDGVEVHNAKTKPREEQYNSTYRVVSVLTVLHQDWLNGKEYKCKVSNKALPAPIEKTISKAKGQPREPQVYTLPPSREEMTKNQVSLTCLVKGFYPSDIAVEWESNGQPENNYKTTPPVLDSDGSFFLYSKLTVDKSRWQQGNVFSCSVMHEALHNHYTQKSLSLSPGK

SEQ ID NO: 37 - protein, 347 aa, synthetic construct
EVQLVESGGGLVQPGGSLRLSCAASGSDVSANGMVWHRQAPGKQREWVAVISSSGSTNYADSVKGRFTISRDNSKNTMYLQMNSLRPEDTAVYYCGVAHYGQTYWGKGTLVTVSSEPKSSDKTHTCPPCPAPEAAGGPSVFLFPPKPKDTLMISRTPEVTCVVVDVSHEDPEVKFNWYVDGVEVHNAKTKPREEQYNSTYRVVSVLTVLHQDWLNGKEYKCKVSNKALPAPIEKTISKAKGQPREPQVYTLPPSREEMTKNQVSLTCLVKGFYPSDIAVEWESNGQPENNYKTTPPVLDSDGSFFLYSKLTVDKSRWQQGNVFSCSVMHEALHNHYTQKSLSLSPGK

SEQ ID NO: 38 - protein, 347 aa, synthetic construct
EVQLVESGGGLVQPGGSLRLSCAASGSDVSANGMVWHRQAPGKQREWVAVISSSGSTNYADSVKGRFTISRDSDKNTMYLQMNSLRPEDTAVYYCGVAHYGQTYWGKGTLVTVSSEPKSSDKTHTCPPCPAPEAAGGPSVFLFPPKPKDTLMISRTPEVTCVVVDVSHEDPEVKFNWYVDGVEVHNAKTKPREEQYNSTYRVVSVLTVLHQDWLNGKEYKCKVSNKALPAPIEKTISKAKGQPREPQVYTLPPSREEMTKNQVSLTCLVKGFYPSDIAVEWESNGQPENNYKTTPPVLDSDGSFFLYSKLTVDKSRWQQGNVFSCSVMHEALHNHYTQKSLSLSPGK

SEQ ID NO: 39 - protein, 347 aa, synthetic construct
QLQLVESGGGLVQPGGSLRLSCAASGSDVSANGMVWHRQAPGKQREWVAVISSSGSTNYADSVKGRFTISRDSDKNTMYLQMNSLRPEDTAVYLCGVAHYGQTYWGKGTLVTVSSEPKSSDKTHTCPPCPAPEAAGGPSVFLFPPKPKDTLMISRTPEVTCVVVDVSHEDPEVKFNWYVDGVEVHNAKTKPREEQYNSTYRVVSVLTVLHQDWLNGKEYKCKVSNKALPAPIEKTISKAKGQPREPQVYTLPPSREEMTKNQVSLTCLVKGFYPSDIAVEWESNGQPENNYKTTPPVLDSDGSFFLYSKLTVDKSRWQQGNVFSCSVMHEALHNHYTQKSLSLSPGK

SEQ ID NO: 40 - protein, 347 aa, synthetic construct
EVQLVESGGGLVQPGGSLRLSCAASGSDVSANGMVWHRQAPGKQREWVAVISSSGSTNYADSVKGRFTISRDSDKNTMYLQMNNLKPEDTAVYLCGVAHYGQTYWGKGTLVTVSSEPKSSDKTHTCPPCPAPEAAGGPSVFLFPPKPKDTLMISRTPEVTCVVVDVSHEDPEVKFNWYVDGVEVHNAKTKPREEQYNSTYRVVSVLTVLHQDWLNGKEYKCKVSNKALPAPIEKTISKAKGQPREPQVYTLPPSREEMTKNQVSLTCLVKGFYPSDIAVEWESNGQPENNYKTTPPVLDSDGSFFLYSKLTVDKSRWQQGNVFSCSVMHEALHNHYTQKSLSLSPGK

SEQ ID NO: 41 - protein, 347 aa, synthetic construct
QLQLVESGGGLVQPGGSLRLSCAASGSDVSANGMVWHRQAPGKGREWVAVISSSGSTNYADSVKGRFTISRDSDKNTMYLQMNSLRPEDTAVYLCGVAHYGQTYWGKGTLVTVSSEPKSSDKTHTCPPCPAPEAAGGPSVFLFPPKPKDTLMISRTPEVTCVVVDVSHEDPEVKFNWYVDGVEVHNAKTKPREEQYNSTYRVVSVLTVLHQDWLNGKEYKCKVSNKALPAPIEKTISKAKGQPREPQVYTLPPSREEMTKNQVSLTCLVKGFYPSDIAVEWESNGQPENNYKTTPPVLDSDGSFFLYSKLTVDKSRWQQGNVFSCSVMHEALHNHYTQKSLSLSPGK

SEQ ID NO: 42 - protein, 347 aa, synthetic construct
QLQLVESGGGLVQPGGSLRLSCAASGSDVSANGMVWHRQAPGKGREWVAVISSSGSTNYADSVKGRFTISRDNSKNTMYLQMNSLRPEDTAVYLCGVAHYGQTYWGKGTLVTVSSEPKSSDKTHTCPPCPAPEAAGGPSVFLFPPKPKDTLMISRTPEVTCVVVDVSHEDPEVKFNWYVDGVEVHNAKTKPREEQYNSTYRVVSVLTVLHQDWLNGKEYKCKVSNKALPAPIEKTISKAKGQPREPQVYTLPPSREEMTKNQVSLTCLVKGFYPSDIAVEWESNGQPENNYKTTPPVLDSDGSFFLYSKLTVDKSRWQQGNVFSCSVMHEALHNHYTQKSLSLSPGK

SEQ ID NO: 43 - protein, 347 aa, synthetic construct
QLQLVESGGGLVQPGGSLRLSCAASGSDVSANGMVWHRQAPGKGREWVAVISSSGSTNYADSVKGRFTISRDNSKNTMYLQMNSLRPEDTAVYYCGVAHYGQTYWGKGTLVTVSSEPKSSDKTHTCPPCPAPEAAGGPSVFLFPPKPKDTLMISRTPEVTCVVVDVSHEDPEVKFNWYVDGVEVHNAKTKPREEQYNSTYRVVSVLTVLHQDWLNGKEYKCKVSNKALPAPIEKTISKAKGQPREPQVYTLPPSREEMTKNQVSLTCLVKGFYPSDIAVEWESNGQPENNYKTTPPVLDSDGSFFLYSKLTVDKSRWQQGNVFSCSVMHEALHNHYTQKSLSLSPGK

SEQ ID NO: 44 - protein, 347 aa, synthetic construct
QLQLVESGGGLVQPGGSLRLSCAASGSDVSANGMVWHRQAPGKGREWVAVISSSGSTNYADSVKGRFTISRDSDKNTMYLQMNSLRPEDTAVYYCGVAHYGQTYWGKGTLVTVSSEPKSSDKTHTCPPCPAPEAAGGPSVFLFPPKPKDTLMISRTPEVTCVVVDVSHEDPEVKFNWYVDGVEVHNAKTKPREEQYNSTYRVVSVLTVLHQDWLNGKEYKCKVSNKALPAPIEKTISKAKGQPREPQVYTLPPSREEMTKNQVSLTCLVKGFYPSDIAVEWESNGQPENNYKTTPPVLDSDGSFFLYSKLTVDKSRWQQGNVFSCSVMHEALHNHYTQKSLSLSPGK

SEQ ID NO: 45 - protein, 347 aa, synthetic construct
QLQLVESGGGLVQPGGSLRLSCAASGSDVSANGMVWHRQAPGKQREWVAVISSSGSTNYADSVKGRFTISRDNSKNTMYLQMNSLRPEDTAVYLCGVAHYGQTYWGKGTLVTVSSEPKSSDKTHTCPPCPAPEAAGGPSVFLFPPKPKDTLMISRTPEVTCVVVDVSHEDPEVKFNWYVDGVEVHNAKTKPREEQYNSTYRVVSVLTVLHQDWLNGKEYKCKVSNKALPAPIEKTISKAKGQPREPQVYTLPPSREEMTKNQVSLTCLVKGFYPSDIAVEWESNGQPENNYKTTPPVLDSDGSFFLYSKLTVDKSRWQQGNVFSCSVMHEALHNHYTQKSLSLSPGK

SEQ ID NO: 46 - protein, 347 aa, synthetic construct
QLQLVESGGGLVQPGGSLRLSCAASGSDVSANGMVWHRQAPGKQREWVAVISSSGSTNYADSVKGRFTISRDNSKNTMYLQMNSLRPEDTAVYYCGVAHYGQTYWGKGTLVTVSSEPKSSDKTHTCPPCPAPEAAGGPSVFLFPPKPKDTLMISRTPEVTCVVVDVSHEDPEVKFNWYVDGVEVHNAKTKPREEQYNSTYRVVSVLTVLHQDWLNGKEYKCKVSNKALPAPIEKTISKAKGQPREPQVYTLPPSREEMTKNQVSLTCLVKGFYPSDIAVEWESNGQPENNYKTTPPVLDSDGSFFLYSKLTVDKSRWQQGNVFSCSVMHEALHNHYTQKSLSLSPGK

SEQ ID NO: 47 - protein, 347 aa, synthetic construct
QLQLVESGGGLVQPGGSLRLSCAASGSDVSANGMVWHRQAPGKQREWVAVISSSGSTNYADSVKGRFTISRDSDKNTMYLQMNSLRPEDTAVYYCGVAHYGQTYWGKGTLVTVSSEPKSSDKTHTCPPCPAPEAAGGPSVFLFPPKPKDTLMISRTPEVTCVVVDVSHEDPEVKFNWYVDGVEVHNAKTKPREEQYNSTYRVVSVLTVLHQDWLNGKEYKCKVSNKALPAPIEKTISKAKGQPREPQVYTLPPSREEMTKNQVSLTCLVKGFYPSDIAVEWESNGQPENNYKTTPPVLDSDGSFFLYSKLTVDKSRWQQGNVFSCSVMHEALHNHYTQKSLSLSPGK

SEQ ID NO: 48 - protein, 450 aa, synthetic construct
EVQLQQPGAELVKPGASVKMSCKASGYTFTSYYMYWVKQRPGQGLEWIGEINPSHGGTNFNEKFKNKATLTVDKSSSTVYMQLSSLTSEDSAVYYCTRGGNYPYFAMDYWGQGTSVTVSSASTKGPSVFPLAPSSKSTSGGTAALGCLVKDYFPEPVTVSWNSGALTSGVHTFPAVLQSSGLYSLSSVVTVPSSSLGTQTYICNVNHKPSNTKVDKRVEPKSCDKTHTCPPCPAPEAAGGPSVFLFPPKPKDTLMISRTPEVTCVVVDVSHEDPEVKFNWYVDGVEVHNAKTKPREEQYNSTYRVVSVLTVLHQDWLNGKEYKCKVSNKALPAPIEKTISKAKGQPREPQVYTLPPSREEMTKNQVSLTCLVKGFYPSDIAVEWESNGQPENNYKTTPPVLDSDGSFFLYSKLTVDKSRWQQGNVFSCSVMHEALHNHYTQKSLSLSPGK

SEQ ID NO: 49 - protein, 214 aa, synthetic construct
DIQMTQTTSSLSASLGDRVTISCRASQDISNYLNWYQQKPDGTVKLLIYYTSRLHSGVPSRFSGSGSGTDYSLTISNLEQEDIATYFCQQGNTLPWTFGGGTKLEIKRTVAAPSVFIFPPSDEQLKSGTASVVCLLNNFYPREAKVQWKVDNALQSGNSQESVTEQDSKDSTYSLSSTLTLSKADYEKHKVYACEVTHQGLSSPVTKSFNRGEC

SEQ ID NO: 50 - protein, 446 aa, synthetic construct
QVQLVQSGAEVKKPGSSVKVSCKASGFNIKDYYMNWVRQAPGQGLEWIGWIDPENANTIYDPKFQGRVTITADESTSTAYMELSSLRSEDTAVYYCYGSSYRFTYWGQGTLVTVSSASTKGPSVFPLAPSSKSTSGGTAALGCLVKDYFPEPVTVSWNSGALTSGVHTFPAVLQSSGLYSLSSVVTVPSSSLGTQTYICNVNHKPSNTKVDKRVEPKSCDKTHTCPPCPAPEAAGGPSVFLFPPKPKDTLMISRTPEVTCVVVDVSHEDPEVKFNWYVDGVEVHNAKTKPREEQYNSTYRVVSVLTVLHQDWLNGKEYKCKVSNKALPAPIEKTISKAKGQPREPQVYTLPPSREEMTKNQVSLTCLVKGFYPSDIAVEWESNGQPENNYKTTPPVLDSDGSFFLYSKLTVDKSRWQQGNVFSCSVMHEALHNHYTQKSLSLSPGK

SEQ ID NO: 51 - protein, 213 aa, synthetic construct
EIVLTQSPATLSLSPGERATLSCSASSSVSYLYWYQQKPGQAPRPWIYLTSNLASGVPARFSGSGSGTDFTLTISSLEPEDFAVYYCQQWSSNPFTFGGGTKVEIKRTVAAPSVFIFPPSDEQLKSGTASVVCLLNNFYPREAKVQWKVDNALQSGNSQESVTEQDSKDSTYSLSSTLTLSKADYEKHKVYACEVTHQGLSSPVTKSFNRGEC